European Patent Application EP 4 112 645 A1, published January 4, 2023. Title: Monoclonal antibodies against claudin-18 for treatment of cancer. Applicant: Astellas Pharma Inc., et al. The sequence listing filed with the application follows.

SEQUENCE LISTING (150 sequences)

SEQ ID NO: 1 - DNA, 786 bp, Homo sapiens
atggccgtgactgcctgtcagggcttggggttcgtggtttcactgattgggattgcgggcatcattgctgccacctgcatggaccagtggagcacccaagacttgtacaacaaccccgtaacagctgttttcaactaccaggggctgtggcgctcctgtgtccgagagagctctggcttcaccgagtgccggggctacttcaccctgctggggctgccagccatgctgcaggcagtgcgagccctgatgatcgtaggcatcgtcctgggtgccattggcctcctggtatccatctttgccctgaaatgcatccgcattggcagcatggaggactctgccaaagccaacatgacactgacctccgggatcatgttcattgtctcaggtctttgtgcaattgctggagtgtctgtgtttgccaacatgctggtgactaacttctggatgtccacagctaacatgtacaccggcatgggtgggatggtgcagactgttcagaccaggtacacatttggtgcggctctgttcgtgggctgggtcgctggaggcctcacactaattgggggtgtgatgatgtgcatcgcctgccggggcctggcaccagaagaaaccaactacaaagccgtttcttatcatgcctcgggccacagtgttgcctacaagcctggaggcttcaaggccagcactggctttgggtccaacaccaaaaacaagaagatatacgatggaggtgcccgcacagaggacgaggtacaatcttatccttccaagcacgactatgtgtaa

SEQ ID NO: 2 - protein, 261 aa, Homo sapiens
MAVTACQGLGFVVSLIGIAGIIAATCMDQWSTQDLYNNPVTAVFNYQGLWRSCVRESSGFTECRGYFTLLGLPAMLQAVRALMIVGIVLGAIGLLVSIFALKCIRIGSMEDSAKANMTLTSGIMFIVSGLCAIAGVSVFANMLVTNFWMSTANMYTGMGGMVQTVQTRYTFGAALFVGWVAGGLTLIGGVMMCIACRGLAPEETNYKAVSYHASGHSVAYKPGGFKASTGFGSNTKNKKIYDGGARTEDEVQSYPSKHDYV

SEQ ID NO: 3 - DNA, 816 bp, Homo sapiens
atggccgtgactgcctgtcagggcttggggttcgtggtttcactgattgggattgcgggcatcattgctgccacctgcatggaccagtggagcacccaagacttgtacaacaaccccgtaacagctgttttcaactaccaggggctgtggcgctcctgtgtccgagagagctctggcttcaccgagtgccggggctacttcaccctgctggggctgccagccatgctgcaggcagtgcgagccctgatgatcgtaggcatcgtcctgggtgccattggcctcctggtatccatctttgccctgaaatgcatccgcattggcagcatggaggactctgccaaagccaacatgacactgacctccgggatcatgttcattgtctcaggtctttgtgcaattgctggagtgtctgtgtttgccaacatgctggtgactaacttctggatgtccacagctaacatgtacaccggcatgggtgaacaaaaactcatctcagaagaggatctggggatggtgcagactgttcagaccaggtacacatttggtgcggctctgttcgtgggctgggtcgctggaggcctcacactaattgggggtgtgatgatgtgcatcgcctgccggggcctggcaccagaagaaaccaactacaaagccgtttcttatcatgcctcgggccacagtgttgcctacaagcctggaggcttcaaggccagcactggctttgggtccaacaccaaaaacaagaagatatacgatggaggtgcccgcacagaggacgaggtacaatcttatccttccaagcacgactatgtgtaa

SEQ ID NO: 4 - protein, 271 aa, Homo sapiens
MAVTACQGLGFVVSLIGIAGIIAATCMDQWSTQDLYNNPVTAVFNYQGLWRSCVRESSGFTECRGYFTLLGLPAMLQAVRALMIVGIVLGAIGLLVSIFALKCIRIGSMEDSAKANMTLTSGIMFIVSGLCAIAGVSVFANMLVTNFWMSTANMYTGMGEQKLISEEDLGMVQTVQTRYTFGAALFVGWVAGGLTLIGGVMMCIACRGLAPEETNYKAVSYHASGHSVAYKPGGFKASTGFGSNTKNKKIYDGGARTEDEVQSYPSKHDYV

SEQ ID NO: 5 - DNA, 813 bp, Homo sapiens
atggccgtgactgcctgtcagggcttggggttcgtggtttcactgattgggattgcgggcatcattgctgccacctgcatggaccagtggagcacccaagacttgtacaacaaccccgtaacagctgttttcaactaccaggggctgtggcgctcctgtgtccgagagagctctggcttcaccgagtgccggggctacttcaccctgtacccatacgacgtgccagactacgcactggggctgccagccatgctgcaggcagtgcgagccctgatgatcgtaggcatcgtcctgggtgccattggcctcctggtatccatctttgccctgaaatgcatccgcattggcagcatggaggactctgccaaagccaacatgacactgacctccgggatcatgttcattgtctcaggtctttgtgcaattgctggagtgtctgtgtttgccaacatgctggtgactaacttctggatgtccacagctaacatgtacaccggcatgggtgggatggtgcagactgttcagaccaggtacacatttggtgcggctctgttcgtgggctgggtcgctggaggcctcacactaattgggggtgtgatgatgtgcatcgcctgccggggcctggcaccagaagaaaccaactacaaagccgtttcttatcatgcctcgggccacagtgttgcctacaagcctggaggcttcaaggccagcactggctttgggtccaacaccaaaaacaagaagatatacgatggaggtgcccgcacagaggacgaggtacaatcttatccttccaagcacgactatgtgtaa

SEQ ID NO: 6 - protein, 270 aa, Homo sapiens
MAVTACQGLGFVVSLIGIAGIIAATCMDQWSTQDLYNNPVTAVFNYQGLWRSCVRESSGFTECRGYFTLYPYDVPDYALGLPAMLQAVRALMIVGIVLGAIGLLVSIFALKCIRIGSMEDSAKANMTLTSGIMFIVSGLCAIAGVSVFANMLVTNFWMSTANMYTGMGGMVQTVQTRYTFGAALFVGWVAGGLTLIGGVMMCIACRGLAPEETNYKAVSYHASGHSVAYKPGGFKASTGFGSNTKNKKIYDGGARTEDEVQSYPSKHDYV

SEQ ID NO: 7 - DNA, 786 bp, Homo sapiens
atgtccaccaccacatgccaagtggtggcgttcctcctgtccatcctggggctggccggctgcatcgcggccaccgggatggacatgtggagcacccaggacctgtacgacaaccccgtcacctccgtgttccagtacgaagggctctggaggagctgcgtgaggcagagttcaggcttcaccgaatgcaggccctatttcaccatcctgggacttccagccatgctgcaggcagtgcgagccctgatgatcgtaggcatcgtcctgggtgccattggcctcctggtatccatctttgccctgaaatgcatccgcattggcagcatggaggactctgccaaagccaacatgacactgacctccgggatcatgttcattgtctcaggtctttgtgcaattgctggagtgtctgtgtttgccaacatgctggtgactaacttctggatgtccacagctaacatgtacaccggcatgggtgggatggtgcagactgttcagaccaggtacacatttggtgcggctctgttcgtgggctgggtcgctggaggcctcacactaattgggggtgtgatgatgtgcatcgcctgccggggcctggcaccagaagaaaccaactacaaagccgtttcttatcatgcctcaggccacagtgttgcctacaagcctggaggcttcaaggccagcactggctttgggtccaacaccaaaaacaagaagatatacgatggaggtgcccgcacagaggacgaggtacaatcttatccttccaagcacgactatgtgtaa

SEQ ID NO: 8 - protein, 261 aa, Homo sapiens
MSTTTCQVVAFLLSILGLAGCIAATGMDMWSTQDLYDNPVTSVFQYEGLWRSCVRQSSGFTECRPYFTILGLPAMLQAVRALMIVGIVLGAIGLLVSIFALKCIRIGSMEDSAKANMTLTSGIMFIVSGLCAIAGVSVFANMLVTNFWMSTANMYTGMGGMVQTVQTRYTFGAALFVGWVAGGLTLIGGVMMCIACRGLAPEETNYKAVSYHASGHSVAYKPGGFKASTGFGSNTKNKKIYDGGARTEDEVQSYPSKHDYV

SEQ ID NO: 9 - DNA, 795 bp, Mus musculus
atggccaccaccacgtgccaggtggtagggcttctcctgtccctcctgggtctggccggctgcatagccgccactgggatggacatgtggagcactcaagacctgtatgacaacccagtcaccgccgtgttccagtatgaagggctctggaggagttgcgtgcaacagagctcggggttcaccgagtgccggccatacttcaccatcctgggccttccagccatgctgcaagctgtacgagccctgatgatcgtgggcattgttctgggggtcatcggtatcctcgtgtccatcttcgccctgaagtgcattcgcattggtagcatggatgactctgccaaggccaagatgactctgacttctgggatcttgttcatcatctccggcatctgtgcaatcattggtgtgtctgtgtttgccaacatgctggtgaccaacttctggatgtccacagctaacatgtacagcggcatgggcggcatgggtggcatggtgcagaccgttcagaccaggtacacctttggtgcagctctgttcgtgggctgggttgctggaggcctcaccctgattgggggagtgatgatgtgcatcgcctgccgtggcctgacaccagatgacagcaacttcaaagctgtgtcttaccatgcctctggccaaaatgttgcctacaggcctggaggctttaaggccagcactggctttgggtccaacaccagaaacaagaagatctacgatgggggtgcccgcacagaagacgatgaacagtctcatcctaccaagtatgactatgtgtag

SEQ ID NO: 10 - DNA, 795 bp, Mus musculus
atgtcggtgaccgcctgccagggcttggggtttgtggtgtcactgatcgggtttgcgggcatcattgcagccacttgtatggaccagtggagcacccaggatttatacaacaacccggtgaccgctgtattcaactaccaagggctatggcgttcatgcgtccgagagagctctggcttcaccgagtgccgaggctacttcaccctgttggggttgccagccatgctgcaagctgtacgagccctgatgatcgtgggcattgttctgggggtcatcggtatcctcgtgtccatcttcgccctgaagtgcattcgcattggtagcatggatgactctgccaaggccaagatgactctgacttctgggatcttgttcatcatctccggcatctgtgcaatcattggtgtgtctgtgtttgccaacatgctggtgaccaacttctggatgtccacagctaacatgtacagcggcatgggcggcatgggtggcatggtgcagaccgttcagaccaggtacacctttggtgcagctctgttcgtgggctgggttgctggaggcctcaccctgattgggggagtgatgatgtgcatcgcctgccgtggcctgacaccagatgacagcaacttcaaagctgtgtcttaccatgcctctggccaaaatgttgcctacaggcctggaggctttaaggccagcactggctttgggtccaacaccagaaacaagaagatctacgatgggggtgcccgcacagaagacgatgaacagtctcatcctaccaagtatgactatgtgtag

SEQ ID NO: 11 - DNA, 21 bp, Artificial
  Description of artificial sequence: Oligonucleotide
tggctctgtgtcgacactgtg

SEQ ID NO: 12 - DNA, 21 bp, Artificial
  Description of artificial sequence: Oligonucleotide
gtgtacatgttagctgtggac

SEQ ID NO: 13 - protein, 55 aa, Homo sapiens
MDMWSTQDLYDNPVTSVFQYEGLWRSCVRQSSGFTECRPYFTILGLPAMLQAVRA

SEQ ID NO: 14 - protein, 153 aa, Homo sapiens
MDMWSTQDLYDNPVTSVFQYEGLWRSCVRQSSGFTECRPYFTILGLPAMLQAVRALMIVGIVLGAIGLLVSIFALKCIRIGSMEDSAKANMTLTSGIMFIVSGLCAIAGVSVFANMLVTNFWMSTANMYTGMGGMVQTVQTRYTFGAALFVGW

SEQ ID NO: 15 - DNA, 390 bp, Homo sapiens
atggagacagacacactcctgctatgggtactgctgctctgggttccaggttccactggtgacgcggcccagccggccaggcgcgcgcgccgtacgaagcttggtaccgagctcggatccactccagtgtggtggaattctgcagatggccgcatggaccagtggagcacccaagacttgtacaacaaccccgtaacagctgttttcaactaccaggggctgtggcgctcctgtgtccgagagagctctggcttcaccgagtgccggggctacttcaccctgctggggctgccagccatgctgcaggcagtgcgagcggccatccagcacagtggcggccgctcgaggagggcccgaacaaaaactcatctcagaagaggatctgaatag

SEQ ID NO: 16 - protein, 129 aa, Homo sapiens
METDTLLLWVLLLWVPGSTGDAAQPARRARRTKLGTELGSTPVWWNSADGRMDQWSTQDLYNNPVTAVFNYQGLWRSCVRESSGFTECRGYFTLLGLPAMLQAVRAAIQHSGGRSRRARTKTHLRRGSE

SEQ ID NO: 17 - DNA, 411 bp, Homo sapiens
atggagacagacacactcctgctatgggtactgctgctctgggttccaggttccactggtgacgcggcccagccggccaggcgcgcgcgccgtacgaagcttggtaccgagctcggatccactccagtgtggtggaattctgcagatggccgcgccctgatgatcgtaggcatcgtcctgggtgccattggcctcctggtatccatctttgccctgaaatgcatccgcattggcagcatggaggactctgccaaagccaacatgacactgacatccgggatcatgttcattgtctcaggtctttgtgcaattgctggagtgtctgtgtttgccaacgcggccatccagcacagtggcggccgctcgaggagggcccgaacaaaaactcatctcagaagaggatctgaatag

SEQ ID NO: 18 - protein, 136 aa, Homo sapiens
METDTLLLWVLLLWVPGSTGDAAQPARRARRTKLGTELGSTPVWWNSADGRALMIVGIVLGAIGLLVSIFALKCIRIGSMEDSAKANMTLTSGIMFIVSGLCAIAGVSVFANAAIQHSGGRSRRARTKTHLRRGSE

SEQ ID NO: 19 - DNA, 531 bp, Homo sapiens
atggagacagacacactcctgctatgggtactgctgctctgggttccaggttccactggtgacgcggcccagccggccaggcgcgccatggaccagtggagcacccaagacttgtacaacaaccccgtaacagctgttttcaactaccaggggctgtggcgctcctgtgtccgagagagctctggcttcaccgagtgccggggctacttcaccctgctggggctgccagccatgctgcaggcagtgcgagccctgatgatcgtaggcatcgtcctgggtgccattggcctcctggtatccatctttgccctgaaatgcatccgcattggcagcatggaggactctgccaaagccaacatgacactgacctccgggatcatgttcattgtctcaggtctttgtgcaattgctggagtgtctgtgtttgccaacatgctggtgactaacttctggatgtccacagctaacatgtacaccggcatgggtgggatggtgcagactgttcagaccaggtacacatttggtgcgtag

SEQ ID NO: 20 - protein, 176 aa, Homo sapiens
METDTLLLWVLLLWVPGSTGDAAQPARRAMDQWSTQDLYNNPVTAVFNYQGLWRSCVRESSGFTECRGYFTLLGLPAMLQAVRALMIVGIVLGAIGLLVSIFALKCIRIGSMEDSAKANMTLTSGIMFIVSGLCAIAGVSVFANMLVTNFWMSTANMYTGMGGMVQTVQTRYTFGA

SEQ ID NO: 21 - protein, 10 aa, Homo sapiens
DQWSTQDLYN

SEQ ID NO: 22 - protein, 11 aa, Homo sapiens
NNPVTAVFNYQ

SEQ ID NO: 23 - protein, 14 aa, Homo sapiens
STQDLYNNPVTAVF

SEQ ID NO: 24 - protein, 12 aa, Homo sapiens
DMWSTQDLYDNP

SEQ ID NO: 25 - protein, 12 aa, Homo sapiens
CRPYFTILGLPA

SEQ ID NO: 26 - protein, 13 aa, Homo sapiens
TNFWMSTANMYTG

SEQ ID NO: 27 - protein, 13 aa, Homo sapiens
DSAKANMTLTSGI

SEQ ID NO: 28 - protein, 55 aa, Homo sapiens
MDQWSTQDLYNNPVTAVFNYQGLWRSCVRESSGFTECRGYFTLLGLPAMLQAVRA

SEQ ID NO: 29 - protein, 24 aa, Homo sapiens
FALKCIRIGSMEDSAKANMTLTSG

SEQ ID NO: 30 - protein, 40 aa, Homo sapiens
ANMLVTNFWMSTANMYTGMGGMVQTVQTRYTFGAALFVGW

SEQ ID NO: 31 - protein, 153 aa, Homo sapiens
MDQWSTQDLYNNPVTAVFNYQGLWRSCVRESSGFTECRGYFTLLGLPAMLQAVRALMIVGIVLGAIGLLVSIFALKCIRIGSMEDSAKANMTLTSGIMFIVSGLCAIAGVSVFANMLVTNFWMSTANMYTGMGGMVQTVQTRYTFGAALFVGW

SEQ ID NO: 32 - DNA, 3359 bp, Homo sapiens
cacaccttcggcagcaggagggcggcagcttctcgcaggcggcagggcgggcggccaggatcatgtccaccaccacatgccaagtggtggcgttcctcctgtccatcctggggctggccggctgcatcgcggccaccgggatggacatgtggagcacccaggacctgtacgacaaccccgtcacctccgtgttccagtacgaagggctctggaggagctgcgtgaggcagagttcaggcttcaccgaatgcaggccctatttcaccatcctgggacttccagccatgctgcaggcagtgcgagccctgatgatcgtaggcatcgtcctgggtgccattggcctcctggtatccatctttgccctgaaatgcatccgcattggcagcatggaggactctgccaaagccaacatgacactgacctccgggatcatgttcattgtctcaggtctttgtgcaattgctggagtgtctgtgtttgccaacatgctggtgactaacttctggatgtccacagctaacatgtacaccggcatgggtgggatggtgcagactgttcagaccaggtacacatttggtgcggctctgttcgtgggctgggtcgctggaggcctcacactaattgggggtgtgatgatgtgcatcgcctgccggggcctggcaccagaagaaaccaactacaaagccgtttcttatcatgcctcaggccacagtgttgcctacaagcctggaggcttcaaggccagcactggctttgggtccaacaccaaaaacaagaagatatacgatggaggtgcccgcacagaggacgaggtacaatcttatccttccaagcacgactatgtgtaatgctctaagacctctcagcacgggcggaagaaactcccggagagctcacccaaaaaacaaggagatcccatctagatttcttcttgcttttgactcacagctggaagttagaaaagcctcgatttcatctttggagaggccaaatggtcttagcctcagtctctgtctctaaatattccaccataaaacagctgagttatttatgaattagaggctatagctcacattttcaatcctctatttctttttttaaatataactttctactctgatgagagaatgtggttttaatctctctctcacattttgatgatttagacagactccccctcttcctcctagtcaataaacccattgatgatctatttcccagcttatccccaagaaaacttttgaaaggaaagagtagacccaaagatgttattttctgctgtttgaattttgtctccccacccccaacttggctagtaataaacacttactgaagaagaagcaataagagaaagatatttgtaatctctccagcccatgatctcggttttcttacactgtgatcttaaaagttaccaaaccaaagtcattttcagtttgaggcaaccaaacctttctactgctgttgacatcttcttattacagcaacaccattctaggagtttcctgagctctccactggagtcctctttctgtcgcgggtcagaaattgtccctagatgaatgagaaaattattttttttaatttaagtcctaaatatagttaaaataaataatgttttagtaaaatgatacactatctctgtgaaatagcctcacccctacatgtggatagaaggaaatgaaaaaataattgctttgacattgtctatatggtactttgtaaagtcatgcttaagtacaaattccatgaaaagctcactgatcctaattctttccctttgaggtctctatggctctgattgtacatgatagtaagtgtaagccatgtaaaaagtaaataatgtctgggcacagtggctcacgcctgtaatcctagcactttgggaggctgaggaggaaggatcacttgagcccagaagttcgagactagcctgggcaacatggagaagccctgtctctacaaaatacagagagaaaaaatcagccagtcatggtggcctacacctgtagtcccagcattccgggaggctgaggtgggaggatcacttgagcccagggaggttggggctgcagtgagccatgatcacaccactgcactccagccaggtgacatagcgagatcctgtctaaaaaaataaaaaataaataatggaacacagcaagtcctaggaagtaggttaaaactaattctttaaaaaaaaaaaaaagttgagcctgaattaaatgtaatgtttccaagtgacaggtatccacatttgcatggttacaagccactgccagttagcagtagcactttcctggcactgtggtcggttttgttttgttttgctttgtttagagacggggtctcactttccaggctggcctcaaactcctgcactcaagcaattcttctaccctggcctcccaagtagctggaattacaggtgtgcgccatcacaactagctggtggtcagttttgttactctgagagctgttcacttctctgaattcacctagagtggttggaccatcagatgtttgggcaaaactgaaagctctttgcaaccacacaccttccctgagcttacatcactgcccttttgagcagaaagtctaaattccttccaagacagtagaattccatcccagtaccaaagccagataggccccctaggaaactgaggtaagagcagtctctaaaaactacccacagcagcattggtgcaggggaacttggccattaggttattatttgagaggaaagtcctcacatcaatagtacatatgaaagtgacctccaaggggattggtgaatactcataaggatcttcaggctgaacagactatgtctggggaaagaacggattatgccccattaaataacaagttgtgttcaagagtcagagcagtgagctcagaggcccttctcactgagacagcaacatttaaaccaaaccagaggaagtatttgtggaactcactgcctcagtttgggtaaaggatgagcagacaagtcaactaaagaaaaaagaaaagcaaggaggagggttgagcaatctagagcatggagtttgttaagtgctctctggatttgagttgaagagcatccatttgagttgaaggccacagggcacaatgagctctcccttctaccaccagaaagtccctggtcaggtctcaggtagtgcggtgtggctcagctgggtttttaattagcgcattctctatccaacatttaattgtttgaaagcctccatatagttagattgtgctttgtaattttgttgttgttgctctatcttattgtatatgcattgagtattaacctgaatgttttgttacttaaatattaaaaacactgttatcctacagtt

SEQ ID NO: 33 - DNA, 849 bp, Mus musculus
gagaacctgcctgtctcttgtcctctccatttgtgtggactctgtgctccatcatgtcggtgaccgcctgccagggcttggggtttgtggtgtcactgatcgggtttgcgggcatcattgcagccacttgtatggaccagtggagcacccaggatttatacaacaacccggtgaccgctgtattcaactaccaagggctatggcgttcatgcgtccgagagagctctggcttcaccgagtgccgaggctacttcaccctgttggggttgccagccatgctgcaagctgtacgagccctgatgatcgtgggcattgttctgggggtcatcggtatcctcgtgtccatcttcgccctgaagtgcattcgcattggtagcatggatgactctgccaaggccaagatgactctgacttctgggatcttgttcatcatctccggcatctgtgcaatcattggtgtgtctgtgtttgccaacatgctggtgaccaacttctggatgtccacagctaacatgtacagcggcatgggcggcatgggtggcatggtgcagaccgttcagaccaggtacaccttcggtgcagctctgttcgtgggctgggttgctggaggcctcaccctgattgggggagtgatgatgtgcatcgcctgccgtggcctgacaccagatgacagcaacttcaaagctgtgtcttaccatgcctctggccaaaatgttgcctacaggcctggaggctttaaggccagcactggctttgggtccaacaccagaaacaagaagatctacgatgggggtgcccgcacagaagacgatgaacagtctcatcctaccaagtatgactatgtgtagt

SEQ ID NO: 34 - DNA, 3350 bp, Homo sapiens
agaattgcgctgtccacttgtcgtgtggctctgtgtcgacactgtgcgccaccatggccgtgactgcctgtcagggcttggggttcgtggtttcactgattgggattgcgggcatcattgctgccacctgcatggaccagtggagcacccaagacttgtacaacaaccccgtaacagctgttttcaactaccaggggctgtggcgctcctgtgtccgagagagctctggcttcaccgagtgccggggctacttcaccctgctggggctgccagccatgctgcaggcagtgcgagccctgatgatcgtaggcatcgtcctgggtgccattggcctcctggtatccatctttgccctgaaatgcatccgcattggcagcatggaggactctgccaaagccaacatgacactgacctccgggatcatgttcattgtctcaggtctttgtgcaattgctggagtgtctgtgtttgccaacatgctggtgactaacttctggatgtccacagctaacatgtacaccggcatgggtgggatggtgcagactgttcagaccaggtacacatttggtgcggctctgttcgtgggctgggtcgctggaggcctcacactaattgggggtgtgatgatgtgcatcgcctgccggggcctggcaccagaagaaaccaactacaaagccgtttcttatcatgcctcaggccacagtgttgcctacaagcctggaggcttcaaggccagcactggctttgggtccaacaccaaaaacaagaagatatacgatggaggtgcccgcacagaggacgaggtacaatcttatccttccaagcacgactatgtgtaatgctctaagacctctcagcacgggcggaagaaactcccggagagctcacccaaaaaacaaggagatcccatctagatttcttcttgcttttgactcacagctggaagttagaaaagcctcgatttcatctttggagaggccaaatggtcttagcctcagtctctgtctctaaatattccaccataaaacagctgagttatttatgaattagaggctatagctcacattttcaatcctctatttctttttttaaatataactttctactctgatgagagaatgtggttttaatctctctctcacattttgatgatttagacagactccccctcttcctcctagtcaataaacccattgatgatctatttcccagcttatccccaagaaaacttttgaaaggaaagagtagacccaaagatgttattttctgctgtttgaattttgtctccccacccccaacttggctagtaataaacacttactgaagaagaagcaataagagaaagatatttgtaatctctccagcccatgatctcggttttcttacactgtgatcttaaaagttaccaaaccaaagtcattttcagtttgaggcaaccaaacctttctactgctgttgacatcttcttattacagcaacaccattctaggagtttcctgagctctccactggagtcctctttctgtcgcgggtcagaaattgtccctagatgaatgagaaaattattttttttaatttaagtcctaaatatagttaaaataaataatgttttagtaaaatgatacactatctctgtgaaatagcctcacccctacatgtggatagaaggaaatgaaaaaataattgctttgacattgtctatatggtactttgtaaagtcatgcttaagtacaaattccatgaaaagctcactgatcctaattctttccctttgaggtctctatggctctgattgtacatgatagtaagtgtaagccatgtaaaaagtaaataatgtctgggcacagtggctcacgcctgtaatcctagcactttgggaggctgaggaggaaggatcacttgagcccagaagttcgagactagcctgggcaacatggagaagccctgtctctacaaaatacagagagaaaaaatcagccagtcatggtggcctacacctgtagtcccagcattccgggaggctgaggtgggaggatcacttgagcccagggaggttggggctgcagtgagccatgatcacaccactgcactccagccaggtgacatagcgagatcctgtctaaaaaaataaaaaataaataatggaacacagcaagtcctaggaagtaggttaaaactaattctttaaaaaaaaaaaaaagttgagcctgaattaaatgtaatgtttccaagtgacaggtatccacatttgcatggttacaagccactgccagttagcagtagcactttcctggcactgtggtcggttttgttttgttttgctttgtttagagacggggtctcactttccaggctggcctcaaactcctgcactcaagcaattcttctaccctggcctcccaagtagctggaattacaggtgtgcgccatcacaactagctggtggtcagttttgttactctgagagctgttcacttctctgaattcacctagagtggttggaccatcagatgtttgggcaaaactgaaagctctttgcaaccacacaccttccctgagcttacatcactgcccttttgagcagaaagtctaaattccttccaagacagtagaattccatcccagtaccaaagccagataggccccctaggaaactgaggtaagagcagtctctaaaaactacccacagcagcattggtgcaggggaacttggccattaggttattatttgagaggaaagtcctcacatcaatagtacatatgaaagtgacctccaaggggattggtgaatactcataaggatcttcaggctgaacagactatgtctggggaaagaacggattatgccccattaaataacaagttgtgttcaagagtcagagcagtgagctcagaggcccttctcactgagacagcaacatttaaaccaaaccagaggaagtatttgtggaactcactgcctcagtttgggtaaaggatgagcagacaagtcaactaaagaaaaaagaaaagcaaggaggagggttgagcaatctagagcatggagtttgttaagtgctctctggatttgagttgaagagcatccatttgagttgaaggccacagggcacaatgagctctcccttctaccaccagaaagtccctggtcaggtctcaggtagtgcggtgtggctcagctgggtttttaattagcgcattctctatccaacatttaattgtttgaaagcctccatatagttagattgtgctttgtaattttgttgttgttgctctatcttattgtatatgcattgagtattaacctgaatgttttgttacttaaatattaaaaacactgttatcctacagtt

SEQ ID NO: 35 - protein, 264 aa, Mus musculus
MSVTACQGLGFVVSLIGFAGIIAATCMDQWSTQDLYNNPVTAVFNYQGLWRSCVRESSGFTECRGYFTLLGLPAMLQAVRALMIVGIVLGVIGILVSIFALKCIRIGSMDDSAKAKMTLTSGILFIISGICAIIGVSVFANMLVTNFWMSTANMYSGMGGMGGMVQTVQTRYTFGAALFVGWVAGGLTLIGGVMMCIACRGLTPDDSNFKAVSYHASGQNVAYRPGGFKASTGFGSNTRNKKIYDGGARTEDDEQSHPTKYDYV

SEQ ID NO: 36 - DNA, 2786 bp, Mus musculus
ggccgggaaccttcccagcaagagggtggtggttgctcctggaagcctgcgcccagcagctgaagccatggccaccaccacgtgccaggtggtagggcttctcctgtccctcctgggtctggccggctgcatagccgccactgggatggacatgtggagcactcaagacctgtatgacaacccagtcaccgccgtgttccagtatgaagggctctggaggagttgcgtgcaacagagctcggggttcaccgagtgccggccatacttcaccatcctgggccttccagccatgctgcaagctgtacgagccctgatgatcgtgggcattgttctgggggtcatcggtatcctcgtgtccatcttcgccctgaagtgcattcgcattggtagcatggatgactctgccaaggccaagatgactctgacttctgggatcttgttcatcatctccggcatctgtgcaatcattggtgtgtctgtgtttgccaacatgctggtgaccaacttctggatgtccacagctaacatgtacagcggcatgggcggcatgggtggcatggtgcagaccgttcagaccaggtacaccttcggtgcagctctgttcgtgggctgggttgctggaggcctcaccctgattgggggagtgatgatgtgcatcgcctgccgtggcctgacaccagatgacagcaacttcaaagctgtgtcttaccatgcctctggccaaaatgttgcctacaggcctggaggctttaaggccagcactggctttgggtccaacaccagaaacaagaagatctacgatgggggtgcccgcacagaagacgatgaacagtctcatcctaccaagtatgactatgtgtagtgctctaagacccgccaacctgtgtgcaggaggaacccttccccaagaagagctcaccccaaagcaacgggagtctaccttgttcccttgttgatttcaactgacatctgaaagttggtaaagcctgattttcatccatagggaggctagacagtcttggccacatgtgtctgcctctaaatatcccatcacaaaacagctgagttatcgtttatgagttagaggccataacactcactttagcccaaccctctgctttttaccgtagactttcttttcatctggtgatggaatggaatttgactcacagactaatactttaatggtttagagaaactttccttcctcgtacttaataagcctgctgatggtcgattttccagcttgaccaccaagggaaattttaaaaggaaaaaaaaatacattaaaaggcattatttcctactcaattgtgccttacccacccccaacttgactgataataataatgaacaccacttaaagaaagaatgccagaggaaagatagttgtgtttccccccagccagtcatctgagtccccctatgtggtgatctagaacattactcgccacagtgattttcaaagaaggcaagcgagcctgttcgctctgctcagcatctgctgattccagcaaggcccttccagagctttccactagaagtcctccttctctcggaagtcagaaattccccctagaagagtaagaaatagattcttttgggtaacctgagtcctaggtatagttataataaatagtatattagcaaaacggtttggtatctcagtgaattagtttcagccttacatatagaaaaagctggggaaaaaaaaagcatcccttgacattgtctatagcgtaagatcctatataaatccaagcttcaacaaaagctcactgagtctaatagttttcttttgaggtctccacggccttagtactcatagatgcagcccctgtttaaaagtaaaaaaattaaagtagcttaaaacgggttctttttttttttttttttttcaaaaaatccaatagagacctgtgtgtctggcatagctacagttactgccaatcgacagggccacttctttggtcctgtaggcagttttgcagttctgacagctgcgccgggcatcaatatgcagaccacacccttctctgtgcttgtaggacgacccgttcaaggagaaagcatgaactccatctccatgtgagcctgaatgctcccaggaaatggagatagggtgctctccaaaacccacctgaacctgaaacagctgtagcgctatgctgtaagagcctggccatcaagttcctatggagaaaaagggcagtccttgcattaatagtgcatatataagtggcctctggggggcagggatgaatattcagtggtggctccgagtatgtacagaccgtctaaggagctgtgttgaccaagagccaggttaatacgcagagtttttcccactgggactacagtgattttagactatactgaagaaggccctctggaaaatcattatctgaaatggcataaagaatgaacagaccaaacaatttaaggggagggggcaggtggaaggagggggaaggaggtagaaataagaatctagggcatgaagattgttaaggttcttggggtccaaatggaaggtcacccctttgaggccatggacacaatgcaccccacccctacccccacctgcccacccaccagaaagtccctggtcggactggaggcagtgagaatcagctgttttcagttagtgggtctcggtgtagcacctggctgtttcaaagcttccccttgctttgccgttttttccgccattgctgtcttgttttctgtgttattaacctccatgttttgtacgttaaatattaaaacactgttaacatccattc

SEQ ID NO: 37 - protein, 264 aa, Mus musculus
MATTTCQVVGLLLSLLGLAGCIAATGMDMWSTQDLYDNPVTAVFQYEGLWRSCVQQSSGFTECRPYFTILGLPAMLQAVRALMIVGIVLGVIGILVSIFALKCIRIGSMDDSAKAKMTLTSGILFIISGICAIIGVSVFANMLVTNFWMSTANMYSGMGGMGGMVQTVQTRYTFGAALFVGWVAGGLTLIGGVMMCIACRGLTPDDSNFKAVSYHASGQNVAYRPGGFKASTGFGSNTRNKKIYDGGARTEDDEQSHPTKYDYV

SEQ ID NO: 38 - DNA, 40 bp, Artificial
  Description of artificial sequence: Oligonucleotide
gagaggatcccgtacggtggctgcaccatctgtcttcatc

SEQ ID NO: 39 - DNA, 37 bp, Artificial
  Description of artificial sequence: Oligonucleotide
gagagcggccgcctaacactctcccctgttgaagctc

SEQ ID NO: 40 - DNA, 324 bp, Artificial
  Description of artificial sequence: PCR product
cgtacggtggctgcaccatctgtcttcatcttcccgccatctgatgagcagttgaaatctggaactgcctctgttgtgtgcctgctgaataacttctatcccagagaggccaaagtacagtggaaggtggataacgccctccaatcgggtaactcccaggagagtgtcacagagcaggacagcaaggacagcacctacagcctcagcagcaccctgacgctgagcaaagcagactacgagaaacacaaagtctacgcctgcgaagtcacccatcagggcctgagctcgcccgtcacaaagagcttcaacaggggagagtgttag

SEQ ID NO: 41 - protein, 107 aa, Artificial [sequence omitted]

SEQ ID NO: 42 - DNA, 34 bp, Artificial
  Description of artificial sequence: Oligonucleotide
gagaaagctttccaccaagggcccatcggtcttc

SEQ ID NO: 43 - DNA, 36 bp, Artificial
  Description of artificial sequence: Oligonucleotide
gagagcggccgctcatttacccggagacagggagag

SEQ ID NO: 44 - DNA, 21 bp, Artificial
  Description of artificial sequence: Oligonucleotide
taccagttgaacttgacctca

SEQ ID NO: 45 - DNA, 981 bp, Artificial
  Description of artificial sequence: PCR product
ggcccatcggtcttccccctggcaccctcctccaagagcacctctgggggcacagcggccctgggctgcctggtcaaggactacttccccgaaccggtgacggtgtcgtggaactcaggcgccctgaccagcggcgtgcacaccttcccggctgtcctacagtcctcaggactctactccctcagcagcgtggtgaccgtgccctccagcagcttgggcacccagacctacatctgcaacgtgaatcacaagcccagcaacaccaaggtggacaagaaagttgagcccaaatcttgtgacaaaactcacacatgcccaccgtgcccagcacctgaactcctggggggaccgtcagtcttcctcttccccccaaaacccaaggacaccctcatgatctcccggacccctgaggtcacatgcgtggtggtggacgtgagccacgaagaccctgaggtcaagttcaactggtacgtggacggcgtggaggtgcataatgccaagacaaagccgcgggaggagcagtacaacagcacgtaccgtgtggtcagcgtcctcaccgtcctgcaccaggactggctgaatggcaaggagtacaagtgcaaggtctccaacaaagccctcccagcccccatcgagaaaaccatctccaaagccaaagggcagccccgagaaccacaggtgtacaccctgcccccatcccgggatgagctgaccaagaaccaggtcagcctgacctgcctggtcaaaggcttctatcccagcgacatcgccgtggagtgggagagcaatgggcagccggagaacaactacaagaccacgcctcccgtgctggactccgacggctccttcttcctctatagcaagctcaccgtggacaagagcaggtggcagcaggggaacgtcttctcatgctccgtgatgcatgaggctctgcacaaccactacacgcagaagagcctctccctgtctccgggtaaatga

SEQ ID NO: 46 - protein, 326 aa, Artificial
  Description of artificial sequence: Translation of PCR product
GPSVFPLAPSSKSTSGGTAALGCLVKDYFPEPVTVSWNSGALTSGVHTFPAVLQSSGLYSLSSVVTVPSSSLGTQTYICNVNHKPSNTKVDKKVEPKSCDKTHTCPPCPAPELLGGPSVFLFPPKPKDTLMISRTPEVTCVVVDVSHEDPEVKFNWYVDGVEVHNAKTKPREEQYNSTYRVVSVLTVLHQDWLNGKEYKCKVSNKALPAPIEKTISKAKGQPREPQVYTLPPSRDELTKNQVSLTCLVKGFYPSDIAVEWESNGQPENNYKTTPPVLDSDGSFFLYSKLTVDKSRWQQGNVFSCSVMHEALHNHYTQKSLSLSPGK

SEQ ID NO: 47 - DNA, 32 bp, Artificial
  Description of artificial sequence: Oligonucleotide
  misc_feature (31)..(32): n is a, c, g, or t
ttttttttttttttttttttttttttttttnn

SEQ ID NO: 48 - DNA, 30 bp, Artificial
  Description of artificial sequence: Oligonucleotide
aagcagtggtatcaacgcagagtacgcggg

SEQ ID NO: 49 - DNA, 26 bp, Artificial
  Description of artificial sequence: Oligonucleotide
ctgctcactggatggtgggaagatgg

SEQ ID NO: 50 - DNA, 25 bp, Artificial
  Description of artificial sequence: Oligonucleotide
gggacagtcactgagctgctcagag

SEQ ID NO: 51 - DNA, 25 bp, Artificial
  Description of artificial sequence: Oligonucleotide
acaggggccagtggatagaccgatg

SEQ ID NO: 52 - DNA, 27 bp, Artificial
  Description of artificial sequence: Oligonucleotide
agccagggaccaagggatagacagatg

SEQ ID NO: 53 - DNA, 45 bp, Artificial
  Description of artificial sequence: Oligonucleotide
gtaatacgactcactatagggcaagcagtggtatcaacgcagagt

SEQ ID NO: 54 - DNA, 22 bp, Artificial
  Description of artificial sequence: Oligonucleotide
gtaatacgactcactatagggc

SEQ ID NO: 55 - DNA, 351 bp, Artificial
  Description of artificial sequence: PCR product
caggttcagctgcagcagtctggagctgagctgatgaagcctggggcctcagtgaagatatcctgcaaggctactggctacacattcagtagctactggatagagtgggtaaagcagaggcctggacatggccttgagtggattggagagattttacctggaagtggtagtactaactacaatgagaagttcaagggcaaggccacattcactgcagatacatcctccaacacagcctacatgcaactcagcagcctgacatctgaggactctgccgtctattactgtgcaagatatgattacccctggtttgcttactggggccaagggactctggtcactgtctctgca

SEQ ID NO: 56 - DNA, 354 bp, Artificial
  Description of artificial sequence: PCR product
cagatccagttggtgcagtctggacctgagctgaagaagcctggagagacagtcaagatctcctgcaaggcttctgggtataccttcacaaactatggaatgaactgggtgaagcaggctccaggaaagggtttaaagtggatgggctggataaacaccaacactggagagccaacatatgctgaagagttcaagggacggtttgccttctctttggaaacctctgccagcactgcctatttgcagatcaacaacctcaaaaatgaggacacggctacatatttctgtgcaagactgggttttggtaatgctatggactactggggtcaaggaacctcagtcaccgtctcctca

SEQ ID NO: 57 - DNA, 348 bp, Artificial
  Description of artificial sequence: PCR product
caggttcagctgcagcagtctggagctgagctggcgaggcccggggcttcagtgaagctgtcctgcaaggcttctggctacaccttcactgactactatataaactgggtgaagcagaggactggacagggccttgagtggattggagagatttatcctggaagtggtaatacttactacaatgagaagttcaagggcaaggccacactgactgcagacaaatcctccagcacagcctacatgcagctcagcagcctgacatctgaggactctgcagtctatttctgtgcaagatcgtatggtgcctttgactactggggccaaggcaccactctcacagtctcctca

SEQ ID NO: 58 - DNA, 354 bp, Artificial
  Description of artificial sequence: PCR product
caggtccaactgcagcagcctggggctgagctggtgaggcctggggcttcagtgaagctgtcctgcaaggcttctggctacaccttcaccagctactggataaactgggtgaagcagaggcctggacaaggccttgagtggatcggaaatatttatccttctgatagttatactaactacaatcaaaagttcaaggacaaggccacattgactgtagacaaatcctccagcacagcctacatgcagctcagcagcccgacatctgaggactctgcggtctattactgtacaagatcgtggaggggtaactcctttgactactggggccaaggcaccactctcacagtctcctca

SEQ ID NO: 59 - DNA, 354 bp, Artificial
  Description of artificial sequence: PCR product
caggttcagctgcagcagtctggacctgagctggtgaagcctggggcttcagtgaagatgtcctgcaaggcttctggatacacattcactgactatgttataagctgggtgaagcagagaactggacagggccttgagtggattggagagatttatcctggaagtggtagtacttactacaatgagaagttcaagggcaaggccacactgactgcagacaaatcctccaacacagcctacatgcagctcagcagcctgacatctgaggactctgcggtctatttctgtgcaagaggggtattactacgggctatggactactggggtcaaggaacctcagtcaccgtctcctca

SEQ ID NO: 60 - DNA, 360 bp, Artificial
  Description of artificial sequence: PCR product
caggttcacctacaacagtctggttctgaactgaggagtcctgggtcttcagtaaagctttcatgcaaggattttgattcagaagtcttcccttttgcttatatgagttggattaggcagaagcctgggcatggatttgaatggattggagacatactcccaagtattggtagaacaatctatggagagaagtttgaggacaaagccacactggatgcagacacagtgtccaacacagcctacttggagctcaacagtctgacatctgaggactctgctatctactactgtgcaaggggggagggctacggtgcctggtttgcttactggggccaagggactctggtcactgtctctgca

SEQ ID NO: 61 - DNA, 339 bp, Artificial
  Description of artificial sequence: PCR product
gacattgtgatgacacagtctccatcctccctgactgtgacagcaggagagaaggtcactatgagctgcaagtccagtcagagtctgttaaacagtggaaatcaaaagaactacttgacctggtaccagcagaaaccagggcagcctcctaaactgttgatctactgggcatccactagggaatctggggtccctgatcgcttcacaggcagtggatctggaacagatttcactctcaccatcagcagtgtgcaggctgaagacctggcagtttattactgtcagaatgattatagttatccgctcacgttcggtgctgggaccaagctggagctgaaa

SEQ ID NO: 62 - DNA, 318 bp, Artificial
  Description of artificial sequence: PCR product
caaattgttctcacccagtctccagcaatcatgtctgcatctccaggggagaaggtcaccataacctgcagtgccagctcaagtgtaagttacatgcactggttccagcagaagccaggcacttctcccaaactctggatttatagcacatccaacctggcttctggagtccctgctcgcttcagtggcagtggatctgggacctcttactctctcacaatcagccgaatggaggctgaagatgctgccacttattactgccagcaaaggagtagttacccacccacgttcggaggggggaccaagctggaaataaaa

SEQ ID NO: 63 - DNA, 321 bp, Artificial
  Description of artificial sequence: PCR product
gacattgtgatgacccagtctcaaaaattcatgtccacatcagtaggagacagggtcagcatcacctgcaaggccagtcagaatgttcgtactgctgtagcctggtatcaacagaaaccagggcagtctcctaaagcactgatttacttggcatccaaccggcacactggagtccctgatcgcttcacaggcagtggatctgggacagatttcactctcaccattagcaatgtgcaatctgaagacctggcagattatttctgtctgcaacattggaattatcctctgacgttcggtggaggcaccaagctggaaatcaaa

SEQ ID NO: 64 - DNA, 339 bp, Artificial
  Description of artificial sequence: PCR product
gacattgtgatgtcacagtctccatcctccctagctgtgtcagttggagagaaggttactatgagctgcaagtccagtcagagccttttatatagtagcaatcaaaagaactacttggcctggtaccagcagaaaccagggcagtctcctaaactgctgatttactgggcatccactagggaatctggggtccctgatcgcttcacaggcagtggatctgggacagatttcactctcaccatcagcagtgtgaaggctgaagacctggcagtttattactgtcagcaatattatagctatccgctcacgttcggtgctgggaccaagctggagctgaaa

SEQ ID NO: 65 - DNA, 339 bp, Artificial
  Description of artificial sequence: PCR product
gacattgtgatgacacagtctccatcctccctgactgtgacagcaggagagaaggtcactatgagctgcaagtccagtcagagtctgttaaacagtggaaatcaaaagaactacttgacctggtaccagcagaaaccagggcagcctcctaaactgttgatctactgggcatccactagggaatctggggtccctgatcgcttcacaggcagtggatctggaacagatttcactctcaccatcagcagtgtgcaggctgaagacctggcagtttattactgtcagaatgattatagttatccattcacgttcggctcggggacaaagttggaaataaaa

SEQ ID NO: 66 - DNA, 336 bp, Artificial
  Description of artificial sequence: PCR product
gacattgtgatgtcacagtctccatcctccctggctgtgtcagcaggagagaaggtcactatgagctgcaaatccagtcagagtctgctcaacagtagaacccgaaagaactacttggcttggtaccagcagaaaccagggcagtctcctaaactgctgatctactgggcatccactagggaatctggggtccctgatcgcttcacaggcagtggatctgggacagatttcactctcaccatcagcagtgtgcaggctgaagacctggcagtttattactgcaagcaatcttataatctgtacacgttcggaggggggaccaagctggaaataaaa

SEQ ID NO: 67 - DNA, 339 bp, Artificial
  Description of artificial sequence: PCR product
gacatcgtgatgtcacagtctccatcctccctagctgtgtcagttggagagaaggttactatgagctgcaagtccagtcagagccttttatatagtagcaatcaaaagaactacttggcctggtaccagcagaaaccagggcagtctcctaaactgctgatttactgggcatccactagggaatctggggtccctgatcgcttcacaggcagtggatctgcaacagatttcactctgaccatcagcagtgtgcaggctgaagaccttgcagattatcactgtggacagggttacagctatccgtacacgttcggaggggggaccaagctggaaataaaa

SEQ ID NO: 68 - DNA, 339 bp, Artificial; identical to SEQ ID NO: 64
  Description of artificial sequence: PCR product

SEQ ID NO: 69 - DNA, 321 bp, Artificial
  Description of artificial sequence: PCR product
aacattgtaatgacccaatctcccaaatccatgtccatgtcagtaggagagagggtcaccttgacctgcaaggccagtgagaatgtggttacttatgtttcctggtatcaacagaaaccagagcagtctcctaaactgctgatatacggggcatccaaccggtacactggggtccccgatcgcttcacaggcagtggatctgcaacagatttcactctcaccatcagcagtgtgaaggctgaagacctggcagtttattactgtcagcaatattatagctatccgctcacgttcggtgctgggaccaagctggagctgaaa

SEQ ID NO: 70 - DNA, 43 bp, Artificial
  Description of artificial sequence: Oligonucleotide
gagaaagcttgccgccaccatggaatggacctgggtctttctc

SEQ ID NO: 71 - DNA, 43 bp, Artificial
  Description of artificial sequence: Oligonucleotide
gagagggcccttggtggaggctgcagagacagtgaccagagtc

SEQ ID NO: 72 - DNA, 47 bp, Artificial
  Description of artificial sequence: Oligonucleotide
gagaaagcttgccgccaccatggattggctgtggaacttgctattcc

SEQ ID NO: 73 - DNA, 44 bp, Artificial
  Description of artificial sequence: Oligonucleotide
gagagggcccttggtggaggctgaggagacggtgactgaggttc

SEQ ID NO: 74 - DNA, 46 bp, Artificial
  Description of artificial sequence: Oligonucleotide
gagaaagcttgccgccaccatggaatggatctggatctttctcttc

SEQ ID NO: 75 - DNA, 44 bp, Artificial
  Description of artificial sequence: Oligonucleotide
gagagggcccttggtggaggctgaggagactgtgagagtggtgc

SEQ ID NO: 76 - DNA, 46 bp, Artificial
  Description of artificial sequence: Oligonucleotide
gagaaagcttgccgccaccatgggatggagctgtatcatcctcttc

SEQ ID NO: 77 - DNA, 43 bp, Artificial
  Description of artificial sequence: Oligonucleotide
gagagggcccttggtggaggctgaggagactgtgagagtggtg

SEQ ID NO: 78 - DNA, 47 bp, Artificial
  Description of artificial sequence: Oligonucleotide
gagaaagcttgccgccaccatggaatggaggatctttctcttcatcc

SEQ ID NO: 79 - DNA, 44 bp, Artificial; identical to SEQ ID NO: 73
  Description of artificial sequence: Oligonucleotide

SEQ ID NO: 80 - DNA, 51 bp, Artificial
  Description of artificial sequence: Oligonucleotide
gagaggtctcaagcttagccaccatggactggatttggatcatgctccatc

SEQ ID NO: 81 - DNA, 44 bp, Artificial
  Description of artificial sequence: Oligonucleotide
gagagggcccttggtggaggctgcagagacagtgaccagagtcc

SEQ ID NO: 82 - DNA, 43 bp, Artificial
  Description of artificial sequence: Oligonucleotide
gagaaagcttgccgccaccatggaatcacagactcaggtcctc

SEQ ID NO: 83 - DNA, 34 bp, Artificial
  Description of artificial sequence: Oligonucleotide
cacacgtacgtttcagctccagcttggtcccagc

SEQ ID NO: 84 - DNA, 46 bp, Artificial
  Description of artificial sequence: Oligonucleotide
gagaaagcttgccgccaccatgcattttcaagtgcagattttcagc

SEQ ID NO: 85 - DNA, 30 bp, Artificial
  Description of artificial sequence: Oligonucleotide
cacacgtacgttttatttccagcttggtcc

SEQ ID NO: 86 - DNA, 44 bp, Artificial
  Description of artificial sequence: Oligonucleotide
gagaaagcttgccgccaccatggagtttcagacccaggtctttg

SEQ ID NO: 87 - DNA, 33 bp, Artificial
  Description of artificial sequence: Oligonucleotide
cacacgtacgtttgatttccagcttggtgcctc

SEQ ID NO: 88 - DNA, 46 bp, Artificial
  Description of artificial sequence: Oligonucleotide
gagaaagcttgccgccaccatggattcacaggcccaggttcttatg

SEQ ID NO: 89 - DNA, 30 bp, Artificial
  Description of artificial sequence: Oligonucleotide
cacacgtacgtttcagctccagcttggtcc

SEQ ID NO: 90 - DNA, 46 bp, Artificial
  Description of artificial sequence: Oligonucleotide
gagaaagcttgccgccaccatggaatcacagactcaggtcctcatg

SEQ ID NO: 91 - DNA, 30 bp, Artificial
  Description of artificial sequence: Oligonucleotide
cacacgtacgttttatttccaactttgtcc

SEQ ID NO: 92 - DNA, 49 bp, Artificial
  Description of artificial sequence: Oligonucleotide
gagaaagcttgccgccaccatggattcacaggcccaggttcttatattg

SEQ ID NO: 93 - DNA, 30 bp, Artificial; identical to SEQ ID NO: 85
  Description of artificial sequence: Oligonucleotide

SEQ ID NO: 94 - DNA, 46 bp, Artificial; identical to SEQ ID NO: 88
  Description of artificial sequence: Oligonucleotide

SEQ ID NO: 95 - DNA, 30 bp, Artificial; identical to SEQ ID NO: 85
  Description of artificial sequence: Oligonucleotide

SEQ ID NO: 96 - DNA, 46 bp, Artificial
  Description of artificial sequence: Oligonucleotide
gagaaagcttgccgccaccatggattcacaggctcaggttcttatg

SEQ ID NO: 97 - DNA, 33 bp, Artificial
  Description of artificial sequence: Oligonucleotide
cacacgtacgtttcagctccagcttggtcccag

SEQ ID NO: 98 - DNA, 41 bp, Artificial
  Description of artificial sequence: Oligonucleotide
gagaaagcttagccaccatggaatcacagactctggtcttc

SEQ ID NO: 99 - DNA, 30 bp, Artificial; identical to SEQ ID NO: 89
  Description of artificial sequence: Oligonucleotide

SEQ ID NO: 100 - DNA, 1401 bp, Artificial
  Description of artificial sequence: chimeric monoclonal antibody
atggaatggacctgggtctttctcttcctcctgtcagtaactgcaggtgtccactcccaggttcagctgcagcagtctggagctgagctgatgaagcctggggcctcagtgaagatatcctgcaaggctactggctacacattcagtagctactggatagagtgggtaaagcagaggcctggacatggccttgagtggattggagagattttacctggaagtggtagtactaactacaatgagaagttcaagggcaaggccacattcactgcagatacatcctccaacacagcctacatgcaactcagcagcctgacatctgaggactctgccgtctattactgtgcaagatatgattacccctggtttgcttactggggccaagggactctggtcactgtctctgcagcctccaccaagggcccatcggtcttccccctggcaccctcctccaagagcacctctgggggcacagcggccctgggctgcctggtcaaggactacttccccgaaccggtgacggtgtcgtggaactcaggcgccctgaccagcggcgtgcacaccttcccggctgtcctacagtcctcaggactctactccctcagcagcgtggtgaccgtgccctccagcagcttgggcacccagacctacatctgcaacgtgaatcacaagcccagcaacaccaaggtggacaagaaagttgagcccaaatcttgtgacaaaactcacacatgcccaccgtgcccagcacctgaactcctggggggaccgtcagtcttcctcttccccccaaaacccaaggacaccctcatgatctcccggacccctgaggtcacatgcgtggtggtggacgtgagccacgaagaccctgaggtcaagttcaactggtacgtggacggcgtggaggtgcataatgccaagacaaagccgcgggaggagcagtacaacagcacgtaccgtgtggtcagcgtcctcaccgtcctgcaccaggactggctgaatggcaaggagtacaagtgcaaggtctccaacaaagccctcccagcccccatcgagaaaaccatctccaaagccaaagggcagccccgagaaccacaggtgtacaccctgcccccatcccgggatgagctgaccaagaaccaggtcagcctgacctgcctggtcaaaggcttctatcccagcgacatcgccgtggagtgggagagcaatgggcagccggagaacaactacaagaccacgcctcccgtgctggactccgacggctccttcttcctctatagcaagctcaccgtggacaagagcaggtggcagcaggggaacgtcttctcatgctccgtgatgcatgaggctctgcacaaccactacacgcagaagagcctctccctgtctccgggtaaatga

SEQ ID NO: 101 - DNA, 1404 bp, Artificial
  Description of artificial sequence: chimeric monoclonal antibody
atggattggctgtggaacttgctattcctgatggcagctgcccaaagtatccaagcacagatccagttggtgcagtctggacctgagctgaagaagcctggagagacagtcaagatctcctgcaaggcttctgggtataccttcacaaactatggaatgaactgggtgaagcaggctccaggaaagggtttaaagtggatgggctggataaacaccaacactggagagccaacatatgctgaagagttcaagggacggtttgccttctctttggaaacctctgccagcactgcctatttgcagatcaacaacctcaaaaatgaggacacggctacatatttctgtgcaagactgggttttggtaatgctatggactactggggtcaaggaacctcagtcaccgtctcctcagcctccaccaagggcccatcggtcttccccctggcaccctcctccaagagcacctctgggggcacagcggccctgggctgcctggtcaaggactacttccccgaaccggtgacggtgtcgtggaactcaggcgccctgaccagcggcgtgcacaccttcccggctgtcctacagtcctcaggactctactccctcagcagcgtggtgaccgtgccctccagcagcttgggcacccagacctacatctgcaacgtgaatcacaagcccagcaacaccaaggtggacaagaaagttgagcccaaatcttgtgacaaaactcacacatgcccaccgtgcccagcacctgaactcctggggggaccgtcagtcttcctcttccccccaaaacccaaggacaccctcatgatctcccggacccctgaggtcacatgcgtggtggtggacgtgagccacgaagaccctgaggtcaagttcaactggtacgtggacggcgtggaggtgcataatgccaagacaaagccgcgggaggagcagtacaacagcacgtaccgtgtggtcagcgtcctcaccgtcctgcaccaggactggctgaatggcaaggagtacaagtgcaaggtctccaacaaagccctcccagcccccatcgagaaaaccatctccaaagccaaagggcagccccgagaaccacaggtgtacaccctgcccccatcccgggatgagctgaccaagaaccaggtcagcctgacctgcctggtcaaaggcttctatcccagcgacatcgccgtggagtgggagagcaatgggcagccggagaacaactacaagaccacgcctcccgtgctggactccgacggctccttcttcctctatagcaagctcaccgtggacaagagcaggtggcagcaggggaacgtcttctcatgctccgtgatgcatgaggctctgcacaaccactacacgcagaagagcctctccctgtctccgggtaaatga

SEQ ID NO: 102 - DNA, 1398 bp, Artificial
  Description of artificial sequence: chimeric monoclonal antibody
atggaatggatctggatctttctcttcatcctctcaggaactgcaggtgtccactcccaggttcagctgcagcagtctggagctgagctggcgaggcccggggcttcagtgaagctgtcctgcaaggcttctggctacaccttcactgactactatataaactgggtgaagcagaggactggacagggccttgagtggattggagagatttatcctggaagtggtaatacttactacaatgagaagttcaagggcaaggccacactgactgcagacaaatcctccagcacagcctacatgcagctcagcagcctgacatctgaggactctgcagtctatttctgtgcaagatcgtatggtgcctttgactactggggccaaggcaccactctcacagtctcctcagcctccaccaagggcccatcggtcttccccctggcaccctcctccaagagcacctctgggggcacagcggccctgggctgcctggtcaaggactacttccccgaaccggtgacggtgtcgtggaactcaggcgccctgaccagcggcgtgcacaccttcccggctgtcctacagtcctcaggactctactccctcagcagcgtggtgaccgtgccctccagcagcttgggcacccagacctacatctgcaacgtgaatcacaagcccagcaacaccaaggtggacaagaaagttgagcccaaatcttgtgacaaaactcacacatgcccaccgtgcccagcacctgaactcctggggggaccgtcagtcttcctcttccccccaaaacccaaggacaccctcatgatctcccggacccctgaggtcacatgcgtggtggtggacgtgagccacgaagaccctgaggtcaagttcaactggtacgtggacggcgtggaggtgcataatgccaagacaaagccgcgggaggagcagtacaacagcacgtaccgtgtggtcagcgtcctcaccgtcctgcaccaggactggctgaatggcaaggagtacaagtgcaaggtctccaacaaagccctcccagcccccatcgagaaaaccatctccaaagccaaagggcagccccgagaaccacaggtgtacaccctgcccccatcccgggatgagctgaccaagaaccaggtcagcctgacctgcctggtcaaaggcttctatcccagcgacatcgccgtggagtgggagagcaatgggcagccggagaacaactacaagaccacgcctcccgtgctggactccgacggctccttcttcctctatagcaagctcaccgtggacaagagcaggtggcagcaggggaacgtcttctcatgctccgtgatgcatgaggctctgcacaaccactacacgcagaagagcctctccctgtctccgggtaaatga

SEQ ID NO: 103 - DNA, 1404 bp, Artificial
  Description of artificial sequence: chimeric monoclonal antibody
atgggatggagctgtatcatcctcttcttggtagcaacagctacaggtgtccactcccaggtccaactgcagcagcctggggctgagctggtgaggcctggggcttcagtgaagctgtcctgcaaggcttctggctacaccttcaccagctactggataaactgggtgaagcagaggcctggacaaggccttgagtggatcggaaatatttatccttctgatagttatactaactacaatcaaaagttcaaggacaaggccacattgactgtagacaaatcctccagcacagcctacatgcagctcagcagcccgacatctgaggactctgcggtctattactgtacaagatcgtggaggggtaactcctttgactactggggccaaggcaccactctcacagtctcctcagcctccaccaagggcccatcggtcttccccctggcaccctcctccaagagcacctctgggggcacagcggccctgggctgcctggtcaaggactacttccccgaaccggtgacggtgtcgtggaactcaggcgccctgaccagcggcgtgcacaccttcccggctgtcctacagtcctcaggactctactccctcagcagcgtggtgaccgtgccctccagcagcttgggcacccagacctacatctgcaacgtgaatcacaagcccagcaacaccaaggtggacaagaaagttgagcccaaatcttgtgacaaaactcacacatgcccaccgtgcccagcacctgaactcctggggggaccgtcagtcttcctcttccccccaaaacccaaggacaccctcatgatctcccggacccctgaggtcacatgcgtggtggtggacgtgagccacgaagaccctgaggtcaagttcaactggtacgtggacggcgtggaggtgcataatgccaagacaaagccgcgggaggagcagtacaacagcacgtaccgtgtggtcagcgtcctcaccgtcctgcaccaggactggctgaatggcaaggagtacaagtgcaaggtctccaacaaagccctcccagcccccatcgagaaaaccatctccaaagccaaagggcagccccgagaaccacaggtgtacaccctgcccccatcccgggatgagctgaccaagaaccaggtcagcctgacctgcctggtcaaaggcttctatcccagcgacatcgccgtggagtgggagagcaatgggcagccggagaacaactacaagaccacgcctcccgtgctggactccgacggctccttcttcctctatagcaagctcaccgtggacaagagcaggtggcagcaggggaacgtcttctcatgctccgtgatgcatgaggctctgcacaaccactacacgcagaagagcctctccctgtctccgggtaaatga

SEQ ID NO: 104 - DNA, 1401 bp, Artificial
  Description of artificial sequence: chimeric monoclonal antibody
atggaatggaggatctttctcttcatcctgtcaggaactgcaggtgtccactcccaggttcagctgcagcagtctggacctgagctggtgaagcctggggcttcagtgaagatgtcctgcaaggcttctggatacacattcactgactatgttataagctgggtgaagcagagaactggacagggccttgagtggattggagagatttatcctggaagtggtagtacttactacaatgagaagttcaagggcaaggccacactgactgcagacaaatcctccaacacagcctacatgcagctcagcagcctgacatctgaggactctgcggtctatttctgtgcaagaggggtattactacgggctatggactactggggtcaaggaacctcagtcaccgtctcctcagcctccaccaagggcccatcggtcttccccctggcaccctcctccaagagcacctctgggggcacagcggccctgggctgcctggtcaaggactacttccccgaaccggtgacggtgtcgtggaactcaggcgccctgaccagcggcgtgcacaccttcccggctgtcctacagtcctcaggactctactccctcagcagcgtggtgaccgtgccctccagcagcttgggcacccagacctacatctgcaacgtgaatcacaagcccagcaacaccaaggtggacaagaaagttgagcccaaatcttgtgacaaaactcacacatgcccaccgtgcccagcacctgaactcctggggggaccgtcagtcttcctcttccccccaaaacccaaggacaccctcatgatctcccggacccctgaggtcacatgcgtggtggtggacgtgagccacgaagaccctgaggtcaagttcaactggtacgtggacggcgtggaggtgcataatgccaagacaaagccgcgggaggagcagtacaacagcacgtaccgtgtggtcagcgtcctcaccgtcctgcaccaggactggctgaatggcaaggagtacaagtgcaaggtctccaacaaagccctcccagcccccatcgagaaaaccatctccaaagccaaagggcagccccgagaaccacaggtgtacaccctgcccccatcccgggatgagctgaccaagaaccaggtcagcctgacctgcctggtcaaaggcttctatcccagcgacatcgccgtggagtgggagagcaatgggcagccggagaacaactacaagaccacgcctcccgtgctggactccgacggctccttcttcctctatagcaagctcaccgtggacaagagcaggtggcagcaggggaacgtcttctcatgctccgtgatgcatgaggctctgcacaaccactacacgcagaagagcctctccctgtctccgggtaaatga

SEQ ID NO: 105 - DNA, 1410 bp, Artificial
  Description of artificial sequence: chimeric monoclonal antibody
atggactggatttggatcatgctccatctgctggcagcagctacaggtatccaatcccaggttcacctacaacagtctggttctgaactgaggagtcctgggtcttcagtaaagctttcatgcaaggattttgattcagaagtcttcccttttgcttatatgagttggattaggcagaagcctgggcatggatttgaatggattggagacatactcccaagtattggtagaacaatctatggagagaagtttgaggacaaagccacactggatgcagacacagtgtccaacacagcctacttggagctcaacagtctgacatctgaggactctgctatctactactgtgcaaggggggagggctacggtgcctggtttgcttactggggccaagggactctggtcactgtctctgcagcctccaccaagggcccatcggtcttccccctggcaccctcctccaagagcacctctgggggcacagcggccctgggctgcctggtcaaggactacttccccgaaccggtgacggtgtcgtggaactcaggcgccctgaccagcggcgtgcacaccttcccggctgtcctacagtcctcaggactctactccctcagcagcgtggtgaccgtgccctccagcagcttgggcacccagacctacatctgcaacgtgaatcacaagcccagcaacaccaaggtggacaagaaagttgagcccaaatcttgtgacaaaactcacacatgcccaccgtgcccagcacctgaactcctggggggaccgtcagtcttcctcttccccccaaaacccaaggacaccctcatgatctcccggacccctgaggtcacatgcgtggtggtggacgtgagccacgaagaccctgaggtcaagttcaactggtacgtggacggcgtggaggtgcataatgccaagacaaagccgcgggaggagcagtacaacagcacgtaccgtgtggtcagcgtcctcaccgtcctgcaccaggactggctgaatggcaaggagtacaagtgcaaggtctccaacaaagccctcccagcccccatcgagaaaaccatctccaaagccaaagggcagccccgagaaccacaggtgtacaccctgcccccatcccgggatgagctgaccaagaaccaggtcagcctgacctgcctggtcaaaggcttctatcccagcgacatcgccgtggagtgggagagcaatgggcagccggagaacaactacaagaccacgcctcccgtgctggactccgacggctccttcttcctctatagcaagctcaccgtggacaagagcaggtggcagcaggggaacgtcttctcatgctccgtgatgcatgaggctctgcacaaccactacacgcagaagagcctctccctgtctccgggtaaatga

SEQ ID NO: 106 - DNA, 723 bp, Artificial
  Description of artificial sequence: chimeric monoclonal antibody
atggaatcacagactcaggtcctcatgtccctgctgttctgggtatctggtacctgtggggacattgtgatgacacagtctccatcctccctgactgtgacagcaggagagaaggtcactatgagctgcaagtccagtcagagtctgttaaacagtggaaatcaaaagaactacttgacctggtaccagcagaaaccagggcagcctcctaaactgttgatctactgggcatccactagggaatctggggtccctgatcgcttcacaggcagtggatctggaacagatttcactctcaccatcagcagtgtgcaggctgaagacctggcagtttattactgtcagaatgattatagttatccgctcacgttcggtgctgggaccaagctggagctgaaacgtacggtggctgcaccatctgtcttcatcttcccgccatctgatgagcagttgaaatctggaactgcctctgttgtgtgcctgctgaataacttctatcccagagaggccaaagtacagtggaaggtggataacgccctccaatcgggtaactcccaggagagtgtcacagagcaggacagcaaggacagcacctacagcctcagcagcaccctgacgctgagcaaagcagactacgagaaacacaaagtctacgcctgcgaagtcacccatcagggcctgagctcgcccgtcacaaagagcttcaacaggggagagtgttag

SEQ ID NO: 107 - DNA, 708 bp, Artificial
  Description of artificial sequence: chimeric monoclonal antibody
atgcattttcaagtgcagattttcagcttcctgctaatcagtgcctcagtcataatgtccagaggacaaattgttctcacccagtctccagcaatcatgtctgcatctccaggggagaaggtcaccataacctgcagtgccagctcaagtgtaagttacatgcactggttccagcagaagccaggcacttctcccaaactctggatttatagcacatccaacctggcttctggagtccctgctcgcttcagtggcagtggatctgggacctcttactctctcacaatcagccgaatggaggctgaagatgctgccacttattactgccagcaaaggagtagttacccacccacgttcggaggggggaccaagctggaaataaaacgtacggtggctgcaccatctgtcttcatcttcccgccatctgatgagcagttgaaatctggaactgcctctgttgtgtgcctgctgaataacttctatcccagagaggccaaagtacagtggaaggtggataacgccctccaatcgggtaactcccaggagagtgtcacagagcaggacagcaaggacagcacctacagcctcagcagcaccctgacgctgagcaaagcagactacgagaaacacaaagtctacgcctgcgaagtcacccatcagggcctgagctcgcccgtcacaaagagcttcaacaggggagagtgttag

SEQ ID NO: 108 - DNA, 705 bp, Artificial
  Description of artificial sequence: chimeric monoclonal antibody
atggagtttcagacccaggtctttgtattcgtgttgctctggttgtctggtgttgatggagacattgtgatgacccagtctcaaaaattcatgtccacatcagtaggagacagggtcagcatcacctgcaaggccagtcagaatgttcgtactgctgtagcctggtatcaacagaaaccagggcagtctcctaaagcactgatttacttggcatccaaccggcacactggagtccctgatcgcttcacaggcagtggatctgggacagatttcactctcaccattagcaatgtgcaatctgaagacctggcagattatttctgtctgcaacattggaattatcctctgacgttcggtggaggcaccaagctggaaatcaaacgtacggtggctgcaccatctgtcttcatcttcccgccatctgatgagcagttgaaatctggaactgcctctgttgtgtgcctgctgaataacttctatcccagagaggccaaagtacagtggaaggtggataacgccctccaatcgggtaactcccaggagagtgtcacagagcaggacagcaaggacagcacctacagcctcagcagcaccctgacgctgagcaaagcagactacgagaaacacaaagtctacgcctgcgaagtcacccatcagggcctgagctcgcccgtcacaaagagcttcaacaggggagagtgttag

SEQ ID NO: 109 - DNA, 723 bp, Artificial
  Description of artificial sequence: chimeric monoclonal antibody
atggattcacaggcccaggttcttatgttactgctgctatgggtatctggtacctgtggggacattgtgatgtcacagtctccatcctccctagctgtgtcagttggagagaaggttactatgagctgcaagtccagtcagagccttttatatagtagcaatcaaaagaactacttggcctggtaccagcagaaaccagggcagtctcctaaactgctgatttactgggcatccactagggaatctggggtccctgatcgcttcacaggcagtggatctgggacagatttcactctcaccatcagcagtgtgaaggctgaagacctggcagtttattactgtcagcaatattatagctatccgctcacgttcggtgctgggaccaagctggagctgaaacgtacggtggctgcaccatctgtcttcatcttcccgccatctgatgagcagttgaaatctggaactgcctctgttgtgtgcctgctgaataacttctatcccagagaggccaaagtacagtggaaggtggataacgccctccaatcgggtaactcccaggagagtgtcacagagcaggacagcaaggacagcacctacagcctcagcagcaccctgacgctgagcaaagcagactacgagaaacacaaagtctacgcctgcgaagtcacccatcagggcctgagctcgcccgtcacaaagagcttcaacaggggagagtgttag

SEQ ID NO: 110 - DNA, 723 bp, Artificial
  Description of artificial sequence: chimeric monoclonal antibody
atggaatcacagactcaggtcctcatgtccctgctgttctgggtatctggtacctgtggggacattgtgatgacacagtctccatcctccctgactgtgacagcaggagagaaggtcactatgagctgcaagtccagtcagagtctgttaaacagtggaaatcaaaagaactacttgacctggtaccagcagaaaccagggcagcctcctaaactgttgatctactgggcatccactagggaatctggggtccctgatcgcttcacaggcagtggatctggaacagatttcactctcaccatcagcagtgtgcaggctgaagacctggcagtttattactgtcagaatgattatagttatccattcacgttcggctcggggacaaagttggaaataaaacgtacggtggctgcaccatctgtcttcatcttcccgccatctgatgagcagttgaaatctggaactgcctctgttgtgtgcctgctgaataacttctatcccagagaggccaaagtacagtggaaggtggataacgccctccaatcgggtaactcccaggagagtgtcacagagcaggacagcaaggacagcacctacagcctcagcagcaccctgacgctgagcaaagcagactacgagaaacacaaagtctacgcctgcgaagtcacccatcagggcctgagctcgcccgtcacaaagagcttcaacaggggagagtgttag

SEQ ID NO: 111 - DNA, 720 bp, Artificial
  Description of artificial sequence: chimeric monoclonal antibody
atggattcacaggcccaggttcttatattgctgctgctatgggtatctggtacctgtggggacattgtgatgtcacagtctccatcctccctggctgtgtcagcaggagagaaggtcactatgagctgcaaatccagtcagagtctgctcaacagtagaacccgaaagaactacttggcttggtaccagcagaaaccagggcagtctcctaaactgctgatctactgggcatccactagggaatctggggtccctgatcgcttcacaggcagtggatctgggacagatttcactctcaccatcagcagtgtgcaggctgaagacctggcagtttattactgcaagcaatcttataatctgtacacgttcggaggggggaccaagctggaaataaaacgtacggtggctgcaccatctgtcttcatcttcccgccatctgatgagcagttgaaatctggaactgcctctgttgtgtgcctgctgaataacttctatcccagagaggccaaagtacagtggaaggtggataacgccctccaatcgggtaactcccaggagagtgtcacagagcaggacagcaaggacagcacctacagcctcagcagcaccctgacgctgagcaaagcagactacgagaaacacaaagtctacgcctgcgaagtcacccatcagggcctgagctcgcccgtcacaaagagcttcaacaggggagagtgttag

SEQ ID NO: 112 - DNA, 723 bp, Artificial
  Description of artificial sequence: chimeric monoclonal antibody
atggattcacaggcccaggttcttatgttactgctgctatgggtatctggtacctgtggggacatcgtgatgtcacagtctccatcctccctagctgtgtcagttggagagaaggttactatgagctgcaagtccagtcagagccttttatatagtagcaatcaaaagaactacttggcctggtaccagcagaaaccagggcagtctcctaaactgctgatttactgggcatccactagggaatctggggtccctgatcgcttcacaggcagtggatctgcaacagatttcactctgaccatcagcagtgtgcaggctgaagaccttgcagattatcactgtggacagggttacagctatccgtacacgttcggaggggggaccaagctggaaataaaacgtacggtggctgcaccatctgtcttcatcttcccgccatctgatgagcagttgaaatctggaactgcctctgttgtgtgcctgctgaataacttctatcccagagaggccaaagtacagtggaaggtggataacgccctccaatcgggtaactcccaggagagtgtcacagagcaggacagcaaggacagcacctacagcctcagcagcaccctgacgctgagcaaagcagactacgagaaacacaaagtctacgcctgcgaagtcacccatcagggcctgagctcgcccgtcacaaagagcttcaacaggggagagtgttag

SEQ ID NO: 113 - DNA, 723 bp, Artificial
  Description of artificial sequence: chimeric monoclonal antibody
atggattcacaggctcaggttcttatgttactgctgctatgggtatctggtacctgtggggacattgtgatgtcacagtctccatcctccctagctgtgtcagttggagagaaggttactatgagctgcaagtccagtcagagccttttatatagtagcaatcaaaagaactacttggcctggtaccagcagaaaccagggcagtctcctaaactgctgatttactgggcatccactagggaatctggggtccctgatcgcttcacaggcagtggatctgggacagatttcactctcaccatcagcagtgtgaaggctgaagacctggcagtttattactgtcagcaatattatagctatccgctcacgttcggtgctgggaccaagctggagctgaaacgtacggtggctgcaccatctgtcttcatcttcccgccatctgatgagcagttgaaatctggaactgcctctgttgtgtgcctgctgaataacttctatcccagagaggccaaagtacagtggaaggtggataacgccctccaatcgggtaactcccaggagagtgtcacagagcaggacagcaaggacagcacctacagcctcagcagcaccctgacgctgagcaaagcagactacgagaaacacaaagtctacgcctgcgaagtcacccatcagggcctgagctcgcccgtcacaaagagcttcaacaggggagagtgttag

SEQ ID NO: 114 - DNA, 705 bp, Artificial
  Description of artificial sequence: chimeric monoclonal antibody
atggaatcacagactctggtcttcatatccatactgctctggttatatggagctgatgggaacattgtaatgacccaatctcccaaatccatgtccatgtcagtaggagagagggtcaccttgacctgcaaggccagtgagaatgtggttacttatgtttcctggtatcaacagaaaccagagcagtctcctaaactgctgatatacggggcatccaaccggtacactggggtccccgatcgcttcacaggcagtggatctgcaacagatttcactctcaccatcagcagtgtgaaggctgaagacctggcagtttattactgtcagcaatattatagctatccgctcacgttcggtgctgggaccaagctggagctgaaacgtacggtggctgcaccatctgtcttcatcttcccgccatctgatgagcagttgaaatctggaactgcctctgttgtgtgcctgctgaataacttctatcccagagaggccaaagtacagtggaaggtggataacgccctccaatcgggtaactcccaggagagtgtcacagagcaggacagcaaggacagcacctacagcctcagcagcaccctgacgctgagcaaagcagactacgagaaacacaaagtctacgcctgcgaagtcacccatcagggcctgagctcgcccgtcacaaagagcttcaacaggggagagtgttag

SEQ ID NO: 115 - protein, 466 aa, Artificial
  Description of artificial sequence: chimeric monoclonal antibody
MEWTWVFLFLLSVTAGVHSQVQLQQSGAELMKPGASVKISCKATGYTFSSYWIEWVKQRPGHGLEWIGEILPGSGSTNYNEKFKGKATFTADTSSNTAYMQLSSLTSEDSAVYYCARYDYPWFAYWGQGTLVTVSAASTKGPSVFPLAPSSKSTSGGTAALGCLVKDYFPEPVTVSWNSGALTSGVHTFPAVLQSSGLYSLSSVVTVPSSSLGTQTYICNVNHKPSNTKVDKKVEPKSCDKTHTCPPCPAPELLGGPSVFLFPPKPKDTLMISRTPEVTCVVVDVSHEDPEVKFNWYVDGVEVHNAKTKPREEQYNSTYRVVSVLTVLHQDWLNGKEYKCKVSNKALPAPIEKTISKAKGQPREPQVYTLPPSRDELTKNQVSLTCLVKGFYPSDIAVEWESNGQPENNYKTTPPVLDSDGSFFLYSKLTVDKSRWQQGNVFSCSVMHEALHNHYTQKSLSLSPGK

SEQ ID NO: 116 - protein, 467 aa, Artificial
  Description of artificial sequence: chimeric monoclonal antibody
MDWLWNLLFLMAAAQSIQAQIQLVQSGPELKKPGETVKISCKASGYTFTNYGMNWVKQAPGKGLKWMGWINTNTGEPTYAEEFKGRFAFSLETSASTAYLQINNLKNEDTATYFCARLGFGNAMDYWGQGTSVTVSSASTKGPSVFPLAPSSKSTSGGTAALGCLVKDYFPEPVTVSWNSGALTSGVHTFPAVLQSSGLYSLSSVVTVPSSSLGTQTYICNVNHKPSNTKVDKKVEPKSCDKTHTCPPCPAPELLGGPSVFLFPPKPKDTLMISRTPEVTCVVVDVSHEDPEVKFNWYVDGVEVHNAKTKPREEQYNSTYRVVSVLTVLHQDWLNGKEYKCKVSNKALPAPIEKTISKAKGQPREPQVYTLPPSRDELTKNQVSLTCLVKGFYPSDIAVEWESNGQPENNYKTTPPVLDSDGSFFLYSKLTVDKSRWQQGNVFSCSVMHEALHNHYTQKSLSLSPGK

SEQ ID NO: 117 - protein, 465 aa, Artificial
  Description of artificial sequence: chimeric monoclonal antibody
MEWIWIFLFILSGTAGVHSQVQLQQSGAELARPGASVKLSCKASGYTFTDYYINWVKQRTGQGLEWIGEIYPGSGNTYYNEKFKGKATLTADKSSSTAYMQLSSLTSEDSAVYFCARSYGAFDYWGQGTTLTVSSASTKGPSVFPLAPSSKSTSGGTAALGCLVKDYFPEPVTVSWNSGALTSGVHTFPAVLQSSGLYSLSSVVTVPSSSLGTQTYICNVNHKPSNTKVDKKVEPKSCDKTHTCPPCPAPELLGGPSVFLFPPKPKDTLMISRTPEVTCVVVDVSHEDPEVKFNWYVDGVEVHNAKTKPREEQYNSTYRVVSVLTVLHQDWLNGKEYKCKVSNKALPAPIEKTISKAKGQPREPQVYTLPPSRDELTKNQVSLTCLVKGFYPSDIAVEWESNGQPENNYKTTPPVLDSDGSFFLYSKLTVDKSRWQQGNVFSCSVMHEALHNHYTQKSLSLSPGK

SEQ ID NO: 118 - protein, 467 aa, Artificial
  Description of artificial sequence: chimeric monoclonal antibody
MGWSCIILFLVATATGVHSQVQLQQPGAELVRPGASVKLSCKASGYTFTSYWINWVKQRPGQGLEWIGNIYPSDSYTNYNQKFKDKATLTVDKSSSTAYMQLSSPTSEDSAVYYCTRSWRGNSFDYWGQGTTLTVSSASTKGPSVFPLAPSSKSTSGGTAALGCLVKDYFPEPVTVSWNSGALTSGVHTFPAVLQSSGLYSLSSVVTVPSSSLGTQTYICNVNHKPSNTKVDKKVEPKSCDKTHTCPPCPAPELLGGPSVFLFPPKPKDTLMISRTPEVTCVVVDVSHEDPEVKFNWYVDGVEVHNAKTKPREEQYNSTYRVVSVLTVLHQDWLNGKEYKCKVSNKALPAPIEKTISKAKGQPREPQVYTLPPSRDELTKNQVSLTCLVKGFYPSDIAVEWESNGQPENNYKTTPPVLDSDGSFFLYSKLTVDKSRWQQGNVFSCSVMHEALHNHYTQKSLSLSPGK

SEQ ID NO: 119 - protein, 466 aa, Artificial
  Description of artificial sequence: chimeric monoclonal antibody
MEWRIFLFILSGTAGVHSQVQLQQSGPELVKPGASVKMSCKASGYTFTDYVISWVKQRTGQGLEWIGEIYPGSGSTYYNEKFKGKATLTADKSSNTAYMQLSSLTSEDSAVYFCARGVLLRAMDYWGQGTSVTVSSASTKGPSVFPLAPSSKSTSGGTAALGCLVKDYFPEPVTVSWNSGALTSGVHTFPAVLQSSGLYSLSSVVTVPSSSLGTQTYICNVNHKPSNTKVDKKVEPKSCDKTHTCPPCPAPELLGGPSVFLFPPKPKDTLMISRTPEVTCVVVDVSHEDPEVKFNWYVDGVEVHNAKTKPREEQYNSTYRVVSVLTVLHQDWLNGKEYKCKVSNKALPAPIEKTISKAKGQPREPQVYTLPPSRDELTKNQVSLTCLVKGFYPSDIAVEWESNGQPENNYKTTPPVLDSDGSFFLYSKLTVDKSRWQQGNVFSCSVMHEALHNHYTQKSLSLSPGK

SEQ ID NO: 120 - protein, 469 aa, Artificial [sequence omitted]

SEQ ID NO: 121 - protein, 240 aa, Artificial
  Description of artificial sequence: chimeric monoclonal antibody
MESQTQVLMSLLFWVSGTCGDIVMTQSPSSLTVTAGEKVTMSCKSSQSLLNSGNQKNYLTWYQQKPGQPPKLLIYWASTRESGVPDRFTGSGSGTDFTLTISSVQAEDLAVYYCQNDYSYPLTFGAGTKLELKRTVAAPSVFIFPPSDEQLKSGTASVVCLLNNFYPREAKVQWKVDNALQSGNSQESVTEQDSKDSTYSLSSTLTLSKADYEKHKVYACEVTHQGLSSPVTKSFNRGEC

SEQ ID NO: 122 - protein, 235 aa, Artificial
  Description of artificial sequence: chimeric monoclonal antibody
MHFQVQIFSFLLISASVIMSRGQIVLTQSPAIMSASPGEKVTITCSASSSVSYMHWFQQKPGTSPKLWIYSTSNLASGVPARFSGSGSGTSYSLTISRMEAEDAATYYCQQRSSYPPTFGGGTKLEIKRTVAAPSVFIFPPSDEQLKSGTASVVCLLNNFYPREAKVQWKVDNALQSGNSQESVTEQDSKDSTYSLSSTLTLSKADYEKHKVYACEVTHQGLSSPVTKSFNRGEC

SEQ ID NO: 123 - protein, 234 aa, Artificial
  Description of artificial sequence: chimeric monoclonal antibody
MEFQTQVFVFVLLWLSGVDGDIVMTQSQKFMSTSVGDRVSITCKASQNVRTAVAWYQQKPGQSPKALIYLASNRHTGVPDRFTGSGSGTDFTLTISNVQSEDLADYFCLQHWNYPLTFGGGTKLEIKRTVAAPSVFIFPPSDEQLKSGTASVVCLLNNFYPREAKVQWKVDNALQSGNSQESVTEQDSKDSTYSLSSTLTLSKADYEKHKVYACEVTHQGLSSPVTKSFNRGEC

SEQ ID NO: 124 - protein, 240 aa, Artificial
  Description of artificial sequence: chimeric monoclonal antibody
MDSQAQVLMLLLLWVSGTCGDIVMSQSPSSLAVSVGEKVTMSCKSSQSLLYSSNQKNYLAWYQQKPGQSPKLLIYWASTRESGVPDRFTGSGSGTDFTLTISSVKAEDLAVYYCQQYYSYPLTFGAGTKLELKRTVAAPSVFIFPPSDEQLKSGTASVVCLLNNFYPREAKVQWKVDNALQSGNSQESVTEQDSKDSTYSLSSTLTLSKADYEKHKVYACEVTHQGLSSPVTKSFNRGEC

SEQ ID NO: 125 - protein, 240 aa, Artificial
  Description of artificial sequence: chimeric monoclonal antibody
MESQTQVLMSLLFWVSGTCGDIVMTQSPSSLTVTAGEKVTMSCKSSQSLLNSGNQKNYLTWYQQKPGQPPKLLIYWASTRESGVPDRFTGSGSGTDFTLTISSVQAEDLAVYYCQNDYSYPFTFGSGTKLEIKRTVAAPSVFIFPPSDEQLKSGTASVVCLLNNFYPREAKVQWKVDNALQSGNSQESVTEQDSKDSTYSLSSTLTLSKADYEKHKVYACEVTHQGLSSPVTKSFNRGEC

SEQ ID NO: 126 - protein, 239 aa, Artificial
  Description of artificial sequence: chimeric monoclonal antibody
MDSQAQVLILLLLWVSGTCGDIVMSQSPSSLAVSAGEKVTMSCKSSQSLLNSRTRKNYLAWYQQKPGQSPKLLIYWASTRESGVPDRFTGSGSGTDFTLTISSVQAEDLAVYYCKQSYNLYTFGGGTKLEIKRTVAAPSVFIFPPSDEQLKSGTASVVCLLNNFYPREAKVQWKVDNALQSGNSQESVTEQDSKDSTYSLSSTLTLSKADYEKHKVYACEVTHQGLSSPVTKSFNRGEC

SEQ ID NO: 127 - protein, 240 aa, Artificial
  Description of artificial sequence: chimeric monoclonal antibody
MDSQAQVLMLLLLWVSGTCGDIVMSQSPSSLAVSVGEKVTMSCKSSQSLLYSSNQKNYLAWYQQKPGQSPKLLIYWASTRESGVPDRFTGSGSATDFTLTISSVQAEDLADYHCGQGYSYPYTFGGGTKLEIKRTVAAPSVFIFPPSDEQLKSGTASVVCLLNNFYPREAKVQWKVDNALQSGNSQESVTEQDSKDSTYSLSSTLTLSKADYEKHKVYACEVTHQGLSSPVTKSFNRGEC

SEQ ID NO: 128 - protein, 240 aa, Artificial; identical to SEQ ID NO: 124
  Description of artificial sequence: chimeric monoclonal antibody

SEQ ID NO: 129 - protein, 234 aa, Artificial
  Description of artificial sequence: chimeric monoclonal antibody
MESQTLVFISILLWLYGADGNIVMTQSPKSMSMSVGERVTLTCKASENVVTYVSWYQQKPEQSPKLLIYGASNRYTGVPDRFTGSGSATDFTLTISSVKAEDLAVYYCQQYYSYPLTFGAGTKLELKRTVAAPSVFIFPPSDEQLKSGTASVVCLLNNFYPREAKVQWKVDNALQSGNSQESVTEQDSKDSTYSLSSTLTLSKADYEKHKVYACEVTHQGLSSPVTKSFNRGEC

SEQ ID NO: 130 - DNA, 18 bp, Artificial
  Description of artificial sequence: Oligonucleotide
ccaagggctatggcgttc

SEQ ID NO: 131 - DNA, 18 bp, Artificial
  Description of artificial sequence: Oligonucleotide
ccgaaggtgtacctggtc

SEQ ID NO: 132 - protein, 117 aa, Artificial
  Description of artificial sequence: Translation of PCR product
QVQLQQSGAELMKPGASVKISCKATGYTFSSYWIEWVKQRPGHGLEWIGEILPGSGSTNYNEKFKGKATFTADTSSNTAYMQLSSLTSEDSAVYYCARYDYPWFAYWGQGTLVTVSA

SEQ ID NO: 133 - protein, 118 aa, Artificial
  Description of artificial sequence: Translation of PCR product
QIQLVQSGPELKKPGETVKISCKASGYTFTNYGMNWVKQAPGKGLKWMGWINTNTGEPTYAEEFKGRFAFSLETSASTAYLQINNLKNEDTATYFCARLGFGNAMDYWGQGTSVTVSS

SEQ ID NO: 134 - protein, 116 aa, Artificial
  Description of artificial sequence: Translation of PCR product
QVQLQQSGAELARPGASVKLSCKASGYTFTDYYINWVKQRTGQGLEWIGEIYPGSGNTYYNEKFKGKATLTADKSSSTAYMQLSSLTSEDSAVYFCARSYGAFDYWGQGTTLTVSS

SEQ ID NO: 135 - protein, 118 aa, Artificial
  Description of artificial sequence: Translation of PCR product
QVQLQQPGAELVRPGASVKLSCKASGYTFTSYWINWVKQRPGQGLEWIGNIYPSDSYTNYNQKFKDKATLTVDKSSSTAYMQLSSPTSEDSAVYYCTRSWRGNSFDYWGQGTTLTVSS

SEQ ID NO: 136 - protein, 118 aa, Artificial
  Description of artificial sequence: Translation of PCR product
QVQLQQSGPELVKPGASVKMSCKASGYTFTDYVISWVKQRTGQGLEWIGEIYPGSGSTYYNEKFKGKATLTADKSSNTAYMQLSSLTSEDSAVYFCARGVLLRAMDYWGQGTSVTVSS

SEQ ID NO: 137 - protein, 120 aa, Artificial
  Description of artificial sequence: Translation of PCR product
QVHLQQSGSELRSPGSSVKLSCKDFDSEVFPFAYMSWIRQKPGHGFEWIGDILPSIGRTIYGEKFEDKATLDADTVSNTAYLELNSLTSEDSAIYYCARGEGYGAWFAYWGQGTLVTVSA

SEQ ID NO: 138 - protein, 113 aa, Artificial
  Description of artificial sequence: Translation of PCR product
DIVMTQSPSSLTVTAGEKVTMSCKSSQSLLNSGNQKNYLTWYQQKPGQPPKLLIYWASTRESGVPDRFTGSGSGTDFTLTISSVQAEDLAVYYCQNDYSYPLTFGAGTKLELK

SEQ ID NO: 139 - protein, 106 aa, Artificial
  Description of artificial sequence: Translation of PCR product
QIVLTQSPAIMSASPGEKVTITCSASSSVSYMHWFQQKPGTSPKLWIYSTSNLASGVPARFSGSGSGTSYSLTISRMEAEDAATYYCQQRSSYPPTFGGGTKLEIK

SEQ ID NO: 140 - protein, 107 aa, Artificial
  Description of artificial sequence: Translation of PCR product
DIVMTQSQKFMSTSVGDRVSITCKASQNVRTAVAWYQQKPGQSPKALIYLASNRHTGVPDRFTGSGSGTDFTLTISNVQSEDLADYFCLQHWNYPLTFGGGTKLEIK

SEQ ID NO: 141 - protein, 113 aa, Artificial
  Description of artificial sequence: Translation of PCR product
DIVMSQSPSSLAVSVGEKVTMSCKSSQSLLYSSNQKNYLAWYQQKPGQSPKLLIYWASTRESGVPDRFTGSGSGTDFTLTISSVKAEDLAVYYCQQYYSYPLTFGAGTKLELK

SEQ ID NO: 142 - protein, 113 aa, Artificial
  Description of artificial sequence: Translation of PCR product
DIVMTQSPSSLTVTAGEKVTMSCKSSQSLLNSGNQKNYLTWYQQKPGQPPKLLIYWASTRESGVPDRFTGSGSGTDFTLTISSVQAEDLAVYYCQNDYSYPFTFGSGTKLEIK

SEQ ID NO: 143 - protein, 112 aa, Artificial
  Description of artificial sequence: Translation of PCR product
DIVMSQSPSSLAVSAGEKVTMSCKSSQSLLNSRTRKNYLAWYQQKPGQSPKLLIYWASTRESGVPDRFTGSGSGTDFTLTISSVQAEDLAVYYCKQSYNLYTFGGGTKLEIK

SEQ ID NO: 144 - protein, 113 aa, Artificial
  Description of artificial sequence: Translation of PCR product
DIVMSQSPSSLAVSVGEKVTMSCKSSQSLLYSSNQKNYLAWYQQKPGQSPKLLIYWASTRESGVPDRFTGSGSATDFTLTISSVQAEDLADYHCGQGYSYPYTFGGGTKLEIK

SEQ ID NO: 145 - protein, 113 aa, Artificial; identical to SEQ ID NO: 141
  Description of artificial sequence: Translation of PCR product

SEQ ID NO: 146 - protein, 107 aa, Artificial
  Description of artificial sequence: Translation of PCR product
NIVMTQSPKSMSMSVGERVTLTCKASENVVTYVSWYQQKPEQSPKLLIYGASNRYTGVPDRFTGSGSATDFTLTISSVKAEDLAVYYCQQYYSYPLTFGAGTKLELK

SEQ ID NO: 147 - DNA, 324 bp, Artificial
  Description of artificial sequence: codon optimized nucleic acid
cgtacggtggccgctcccagcgtgttcatcttcccccccagcgacgagcagctgaagtccggcaccgccagcgtggtgtgcctgctgaacaacttctacccccgggaggccaaggtgcagtggaaggtggacaacgccctgcagagcggcaacagccaggagagcgtcaccgagcaggacagcaaggactccacctacagcctgagcagcaccctgaccctgagcaaggccgactacgagaagcacaaggtgtacgcctgcgaggtgacccaccagggcctgtccagccccgtgaccaagagcttcaacaggggcgagtgctag

SEQ ID NO: 148 - protein, 107 aa, Artificial [sequence omitted]

SEQ ID NO: 149 - DNA, 981 bp, Artificial
  Description of artificial sequence: codon optimized nucleic acid
ggcccaagcgtgttccccctggcccccagcagcaagagcaccagcggcggcacagccgccctgggctgcctggtgaaggactacttccccgagcccgtgaccgtgagctggaacagcggagccctgacctccggcgtgcacaccttccccgccgtgctgcagagcagcggcctgtacagcctgagcagcgtggtgaccgtgcccagcagcagcctgggcacccagacctacatctgcaacgtgaaccacaagcccagcaacaccaaggtggacaagagagtggagcccaagagctgcgacaagacccacacctgccccccctgcccagccccagagctgctgggcggacccagcgtgttcctgttcccccccaagcccaaggacaccctgatgatcagcaggacccccgaggtgacctgcgtggtggtggacgtgagccacgaggacccagaggtgaagttcaactggtacgtggacggcgtggaggtgcacaacgccaagaccaagcccagagaggagcagtacaacagcacctacagggtggtgtccgtgctgaccgtgctgcaccaggactggctgaacggcaaggaatacaagtgcaaggtctccaacaaggccctgccagcccccatcgaaaagaccatcagcaaggccaagggccagccacgggagccccaggtgtacaccctgccccccagccgggaggagatgaccaagaaccaggtgtccctgacctgtctggtgaagggcttctaccccagcgacatcgccgtggagtgggagagcaacggccagcccgagaacaactacaagaccacccccccagtgctggacagcgacggcagcttcttcctgtacagcaagctgaccgtggacaagtccaggtggcagcagggcaacgtgttcagctgcagcgtgatgcacgaggccctgcacaaccactacacccagaagtccctgagcctgagccccggcaagtag

SEQ ID NO: 150 - protein, 326 aa, Artificial
  Description of artificial sequence: codon optimized protein
GPSVFPLAPSSKSTSGGTAALGCLVKDYFPEPVTVSWNSGALTSGVHTFPAVLQSSGLYSLSSVVTVPSSSLGTQTYICNVNHKPSNTKVDKRVEPKSCDKTHTCPPCPAPELLGGPSVFLFPPKPKDTLMISRTPEVTCVVVDVSHEDPEVKFNWYVDGVEVHNAKTKPREEQYNSTYRVVSVLTVLHQDWLNGKEYKCKVSNKALPAPIEKTISKAKGQPREPQVYTLPPSREEMTKNQVSLTCLVKGFYPSDIAVEWESNGQPENNYKTTPPVLDSDGSFFLYSKLTVDKSRWQQGNVFSCSVMHEALHNHYTQKSLSLSPGK